European Patent Specification EP 3 013 956 B1, published March 1, 2023. Title: SUBTILASE VARIANTS AND POLYNUCLEOTIDES ENCODING SAME. Applicant: Novozymes A/S. The sequence listing filed with the application follows.

SEQUENCE LISTING (4 sequences)

SEQ ID NO: 1 - DNA, 1149 bp, Bacillus amyloliquefaciens
  CDS (1)..(1146)
  sig_peptide (1)..(90)
  mat_peptide (322)..(1146)
atgagaggcaaaaaagtatggatcagtttgctgtttgctttagcgttaatctttacgatggcgttcggcagcacatcctctgcccaggcggcagggaaatcaaacggggaaaagaaatatattgtcgggtttaaacagacaatgagcacgatgagcgccgctaagaagaaagatgtcatttctgaaaaaggcgggaaagtgcaaaagcaattcaaatatgtagacgcagcttcagctacattaaacgaaaaagctgtaaaagaattgaaaaaagacccgagcgtcgcttacgttgaagaagatcacgtagcacatgcgtacgcgcagtccgtgccttacggcgtatcacaaattaaagcccctgctctgcactctcaaggctacactggatcaaatgttaaagtagcggttatcgacagcggtatcgattcttctcatcctgatttaaaggtagcaggcggagccagcatggttccttctgaaacaaatcctttccaagacaacaactctcacggaactcacgttgccggcacagttgcggctcttaataactcaatcggtgtattaggcgttgcgccaagcgcatcactttacgctgtaaaagttctcggtgctgacggttccggccaatacagctggatcattaacggaatcgagtgggcgatcgcaaacaatatggacgttattaacatgagcctcggcggaccttctggttctgctgctttaaaagcggcagttgataaagccgttgcatccggcgtcgtagtcgttgcggcagccggtaacgaaggcacttccggcagctcaagcacagtgggctaccctggtaaatacccttctgtcattgcagtaggcgctgttgacagcagcaaccaaagagcatctttctcaagcgtaggacctgagcttgatgtcatggcacctggcgtatctatccaaagcacgcttcctggaaacaaatacggggcgtacaacggtacgtcaatggcatctccgcacgttgccggagcggctgctttgattctttctaagcacccgaactggacaaacactcaagtccgcagcagtttagaaaacaccactacaaaacttggtgattctttctactatggaaaagggctgatcaacgtacaggcggcagctcagtaa

SEQ ID NO: 2 - protein, 382 aa, Bacillus amyloliquefaciens
MRGKKVWISLLFALALIFTMAFGSTSSAQAAGKSNGEKKYIVGFKQTMSTMSAAKKKDVISEKGGKVQKQFKYVDAASATLNEKAVKELKKDPSVAYVEEDHVAHAYAQSVPYGVSQIKAPALHSQGYTGSNVKVAVIDSGIDSSHPDLKVAGGASMVPSETNPFQDNNSHGTHVAGTVAALNNSIGVLGVAPSASLYAVKVLGADGSGQYSWIINGIEWAIANNMDVINMSLGGPSGSAALKAAVDKAVASGVVVVAAAGNEGTSGSSSTVGYPGKYPSVIAVGAVDSSNQRASFSSVGPELDVMAPGVSIQSTLPGNKYGAYNGTSMASPHVAGAAALILSKHPNWTNTQVRSSLENTTTKLGDSFYYGKGLINVQAAAQ

SEQ ID NO: 3 - DNA, 1143 bp, Bacillus lentus
  CDS (1)..(1140)
  sig_peptide (1)..(81)
  mat_peptide (334)..(1140)
atgaagaaaccgttggggaaaattgtcgcaagcaccgcactactcatttctgttgcttttagttcatcgatcgcatcggctgctgaagaagcaaaagaaaaatatttaattggctttaatgagcaggaagctgtcagtgagtttgtagaacaagtagaggcaaatgacgaggtcgccattctctctgaggaagaggaagtcgaaattgaattgcttcatgaatttgaaacgattcctgttttatccgttgagttaagcccagaagatgtggacgcgcttgaactcgatccagcgatttcttatattgaagaggatgcagaagtaacgacaatggcgcaatcggtaccatggggaattagccgtgtgcaagccccagctgcccataaccgtggattgacaggttctggtgtaaaagttgctgtcctcgatacagggatatccactcatccagatctaaatattcgtggtggcgcaagctttgtaccaggggaaccgtcgactcaagatgggaatgggcatggcacgcatgtggccgggacgatcgctgctttaaacaattcgattggcgttcttggcgtagctcctagcgctgagctatacgctgttaaagtcctaggggcgagcggttcaggttcggtcagctcgattgcccaaggattggaatgggcagggaacaatggcatgcacgttgctaatttgagtttaggaagcccttcgccaagtgccacactcgagcaagctgttaatagcgcgacttctagaggcgttcttgttgtagcggcatctgggaattcaggtgcaggctcaatcagctatccggcgcgctatgcgaacgcaatggcagtcggagctactgatcaaaacaacaaccgcgctagcttttcacagtatggcgcaggccttgacattgtcgcacccggggtaaacgtgcagagcacatacccaggttcaacatatgccagcttaaacggtacatcgatggctactcctcatgttgcaggtgcggccgcccttgttaaacaaaagaacccatcttggtctaatgtacaaattcgaaatcatctaaagaatacggcaactagtttaggaagcacgaacttgtatggaagcggacttgttaacgcagaagcggcaacgcgttaa

SEQ ID NO: 4 - protein, 380 aa, Bacillus lentus
MKKPLGKIVASTALLISVAFSSSIASAAEEAKEKYLIGFNEQEAVSEFVEQVEANDEVAILSEEEEVEIELLHEFETIPVLSVELSPEDVDALELDPAISYIEEDAEVTTMAQSVPWGISRVQAPAAHNRGLTGSGVKVAVLDTGISTHPDLNIRGGASFVPGEPSTQDGNGHGTHVAGTIAALNNSIGVLGVAPSAELYAVKVLGASGSGSVSSIAQGLEWAGNNGMHVANLSLGSPSPSATLEQAVNSATSRGVLVVAASGNSGAGSISYPARYANAMAVGATDQNNNRASFSQYGAGLDIVAPGVNVQSTYPGSTYASLNGTSMATPHVAGAAALVKQKNPSWSNVQIRNHLKNTATSLGSTNLYGSGLVNAEAATR